European Patent Specification EP 4 081 650 B1, published November 29, 2023. Title: Protein and peptide fingerprinting and sequencing by nanopore translocation of peptide oligonucleotide complexes. Applicant: Technische Universiteit Delft. Application NL2024579. The sequence listing filed with the application follows.

SEQUENCE LISTING (5 sequences)

SEQ ID NO: 1 - DNA, 35 bp, Artificial Sequence
  Oligonucleotide for examples 1 and 2
  modified_base 3..4: /mod_base="OTHER" /note="Abasic site; DNA backbone only"
ctnntgtagtcgtcgttgtgcagtcgttcgtagcc

SEQ ID NO: 2 - protein, 30 aa, Artificial Sequence
  Peptide for examples 1 and 2
DDEDEEEDDDEDEDEEDDEDEDEEEEDDDD

SEQ ID NO: 3 - DNA, 22 bp, Artificial Sequence
  Oligonucleotide for example 3
ttcgaaccgtctgatgtagtcg

SEQ ID NO: 4 - protein, 23 aa, Artificial Sequence
  Peptide for example 3
DDEDEDEEDDEDEWEEEEDDDDC

SEQ ID NO: 5 - DNA, 42 bp, Artificial Sequence
  complementary oligonucleotide Fig. 2
acgactgcacaacgacgactactttttttttttttttttttt